European Patent Application EP 4 324 847 A1, published February 21, 2024. Title: INTERLEUKIN-2 MUTANT AND APPLICATION THEREOF. Applicant: SUZHOU FORLONG BIOTECHNOLOGY CO., LTD. Application EP 22787516.8. The sequence listing filed with the application follows.

SEQUENCE LISTING (42 sequences)

SEQ ID NO: 1 - DNA, 399 bp, Artificial Sequence
gccccaactagcagcagcaccaaaaaaactcagctgcagctggaacatctgctgctggatctgcagatgattctgaatggcattaacaactataaaaacccannbctgactnnbatgctgaccnnbnnbtttnnbatgccaaaaaaagccactgaactgaaacatctgcagtgcctggaagaannbctgaaaccactggaagaagtgctgaacnnbgcacagagcaaaaactttcatctgagaccaagagatctgattagcaacattaatgtgattgtgctggaactgaaaggcagtgaaaccacctttatgtgtgaatatgcagatgaaactgccaccattgtggaatttctgaacagatggattaccttttgtcagagcattattagcaccctgacc

SEQ ID NO: 2 - DNA, 399 bp, Artificial Sequence
gccccaactagcagcagcaccaaaaaaactcagctgcagctggaacatctgctgctggatctgcagatgattctgaatggcattaacaactataaaaacccactgctgactgacatgctgaccttgcatttttacatgccaaaaaaagccactgaactgaaacatctgcagtgcctggaagaagagctgaaaccactggaagaagtgctgaactttgcacagagcaaaaactttcatctgagaccaagagatctgattagcaacattaatgtgattgtgctggaactgaaaggcagtgaaaccacctttatgtgtgaatatgcagatgaaactgccaccattgtggaatttctgaacagatggattaccttttgtcagagcattattagcaccctgacc

SEQ ID NO: 3 - DNA, 399 bp, Artificial Sequence
gccccaactagcagcagcaccaaaaaaactcagctgcagctggaacatctgctgctggatctgcagatgattctgaatggcattaacaactataaaaacccaatgctgactgatatgctgaccgtgggcttttttatgccaaaaaaagccactgaactgaaacatctgcagtgcctggaagaagagctgaaaccactggaagaagtgctgaactttgcacagagcaaaaactttcatctgagaccaagagatctgattagcaacattaatgtgattgtgctggaactgaaaggcagtgaaaccacctttatgtgtgaatatgcagatgaaactgccaccattgtggaatttctgaacagatggattaccttttgtcagagcattattagcaccctgacc

SEQ ID NO: 4 - DNA, 399 bp, Artificial Sequence
gccccaactagcagcagcaccaaaaaaactcagctgcagctggaacatctgctgctggatctgcagatgattctgaatggcattaacaactataaaaacccagagctgactgacatgctgacctttaaattttatatgccaaaaaaagccactgaactgaaacatctgcagtgcctggaagaagagctgaaaccactggaagaagtgctgaacgctgcacagagcaaaaactttcatctgagaccaagagatctgattagcaacattaatgtgattgtgctggaactgaaaggcagtgaaaccacctttatgtgtgaatatgcagatgaaactgccaccattgtggaatttctgaacagatggattaccttttgtcagagcattattagcaccctgacc

SEQ ID NO: 5 - DNA, 399 bp, Artificial Sequence
gccccaactagcagcagcaccaaaaaaactcagctgcagctggaacatctgctgctggatctgcagatgattctgaatggcattaacaactataaaaacccagggctgactgatatgctgaccattcagttttttatgccaaaaaaagccactgaactgaaacatctgcagtgcctggaagaagagctgaaaccactggaagaagtgctgaactttgcacagagcaaaaactttcatctgagaccaagagatctgattagcaacattaatgtgattgtgctggaactgaaaggcagtgaaaccacctttatgtgtgaatatgcagatgaaactgccaccattgtggaatttctgaacagatggattaccttttgtcagagcattattagcaccctgacc

SEQ ID NO: 6 - DNA, 399 bp, Artificial Sequence
gccccaactagcagcagcaccaaaaaaactcagctgcagctggaacatctgctgctggatctgcagatgattctgaatggcattaacaactataaaaacccaagcctgactgacatgctgacccttcagttttatatgccaaaaaaagccactgaactgaaacatctgcagtgcctggaagaagagctgaaaccactggaagaagtgctgaactttgcacagagcaaaaactttcatctgagaccaagagatctgattagcaacattaatgtgattgtgctggaactgaaaggcagtgaaaccacctttatgtgtgaatatgcagatgaaactgccaccattgtggaatttctgaacagatggattaccttttgtcagagcattattagcaccctgacc

SEQ ID NO: 7 - DNA, 399 bp, Artificial Sequence
gccccaactagcagcagcaccaaaaaaactcagctgcagctggaacatctgctgctggatctgcagatgattctgaatggcattaacaactataaaaacccagatctgactgatatgctgaccctccggttttttatgccaaaaaaagccactgaactgaaacatctgcagtgcctggaagaagagctgaaaccactggaagaagtgctgaactttgcacagagcaaaaactttcatctgagaccaagagatctgattagcaacattaatgtgattgtgctggaactgaaaggcagtgaaaccacctttatgtgtgaatatgcagatgaaactgccaccattgtggaatttctgaacagatggattaccttttgtcagagcattattagcaccctgacc

SEQ ID NO: 8 - DNA, 399 bp, Artificial Sequence
gccccaactagcagcagcaccaaaaaaactcagctgcagctggaacatctgctgctggatctgcagatgattctgaatggcattaacaactataaaaacccagatctgactgagatgctgacctttaaattttatatgccaaaaaaagccactgaactgaaacatctgcagtgcctggaagaagaactgaaaccactggaagaagtgctgaaccaggcacagagcaaaaactttcatctgagaccaagagatctgattagcaacattaatgtgattgtgctggaactgaaaggcagtgaaaccacctttatgtgtgaatatgcagatgaaactgccaccattgtggaatttctgaacagatggattaccttttgtcagagcattattagcaccctgacc

SEQ ID NO: 9 - DNA, 399 bp, Artificial Sequence
gccccaactagcagcagcaccaaaaaaactcagctgcagctggaacatctgctgctggatctgcagatgattctgaatggcattaacaactataaaaacccatacctgactgacatgctgaccctgggtttttatatgccaaaaaaagccactgaactgaaacatctgcagtgcctggaagaagagctgaaaccactggaagaagtgctgaacttcgcacagagcaaaaactttcatctgagaccaagagatctgattagcaacattaatgtgattgtgctggaactgaaaggcagtgaaaccacctttatgtgtgaatatgcagatgaaactgccaccattgtggaatttctgaacagatggattaccttttgtcagagcattattagcaccctgacc

SEQ ID NO: 10 - DNA, 399 bp, Artificial Sequence
gccccaactagcagcagcaccaaaaaaactcagctgcagctggaacatctgctgctggatctgcagatgattctgaatggcattaacaactataaaaacccagggctgactgacatgctgacctttaacttttatatgccaaaaaaagccactgaactgaaacatctgcagtgcctggaagaagagctgaaaccactggaagaagtgctgaacttcgcacagagcaaaaactttcatctgagaccaagagatctgattagcaacattaatgtgattgtgctggaactgaaaggcagtgaaaccacctttatgtgtgaatatgcagatgaaactgccaccattgtggaatttctgaacagatggattaccttttgtcagagcattattagcaccctgacc

SEQ ID NO: 11 - DNA, 399 bp, Artificial Sequence
gccccaactagcagcagcaccaaaaaaactcagctgcagctggaacatctgctgctggatctgcagatgattctgaatggcattaacaactataaaaacccagggctgactgacatgctgacctactcctttgacatgccaaaaaaagccactgaactgaaacatctgcagtgcctggaagaagagctgaaaccactggaagaagtgctgaacttggcacagagcaaaaactttcatctgagaccaagagatctgattagcaacattaatgtgattgtgctggaactgaaaggcagtgaaaccacctttatgtgtgaatatgcagatgaaactgccaccattgtggaatttctgaacagatggattaccttttgtcagagcattattagcaccctgacc

SEQ ID NO: 12 - DNA, 399 bp, Artificial Sequence
gccccaactagcagcagcaccaaaaaaactcagctgcagctggaacatctgctgctggatctgcagatgattctgaatggcattaacaactataaaaacccagatctgactgagatgctgacctttaaattttatatgccaaaaaaagccactgaactgaaacatctgcagtgcctggaagaagaactgaaaccactggaagaagtgctgaactcggcacagagcaaaaactttcatctgagaccaagagatctgattagcaacattaatgtgattgtgctggaactgaaaggcagtgaaaccacctttatgtgtgaatatgcagatgaaactgccaccattgtggaatttctgaacagatggattaccttttgtcagagcattattagcaccctgacc

SEQ ID NO: 13 - DNA, 399 bp, Artificial Sequence
gccccaactagcagcagcaccaaaaaaactcagctgcagctggaacatctgctgctggatctgcagatgattctgaatggcattaacaactataaaaacccagagctgactgagatgctgacctttaaattttatatgccaaaaaaagccactgaactgaaacatctgcagtgcctggaagaagaactgaaaccactggaagaagtgctgaacgctgcacagagcaaaaactttcatctgagaccaagagatctgattagcaacattaatgtgattgtgctggaactgaaaggcagtgaaaccacctttatgtgtgaatatgcagatgaaactgccaccattgtggaatttctgaacagatggattaccttttgtcagagcattattagcaccctgacc

SEQ ID NO: 14 - DNA, 399 bp, Artificial Sequence
gccccaactagcagcagcaccaaaaaaactcagctgcagctggaacatctgctgctggatctgcagatgattctgaatggcattaacaactataaaaacccagagctgactgacatgctgacctttaaattttatatgccaaaaaaagccactgaactgaaacatctgcagtgcctggaagaagaactgaaaccactggaagaagtgctgaacggtgcacagagcaaaaactttcatctgagaccaagagatctgattagcaacattaatgtgattgtgctggaactgaaaggcagtgaaaccacctttatgtgtgaatatgcagatgaaactgccaccattgtggaatttctgaacagatggattaccttttgtcagagcattattagcaccctgacc

SEQ ID NO: 15 - DNA, 399 bp, Artificial Sequence
gccccaactagcagcagcaccaaaaaaactcagctgcagctggaacatctgctgctggatctgcagatgattctgaatggcattaacaactataaaaacccagatctgactgatatgctgacctttaaattttatatgccaaaaaaagccactgaactgaaacatctgcagtgcctggaagaagaactgaaaccactggaagaagtgctgaacgcggcacagagcaaaaactttcatctgagaccaagagatctgattagcaacattaatgtgattgtgctggaactgaaaggcagtgaaaccacctttatgtgtgaatatgcagatgaaactgccaccattgtggaatttctgaacagatggattaccttttgtcagagcattattagcaccctgacc

SEQ ID NO: 16 - DNA, 399 bp, Artificial Sequence
gccccaactagcagcagcaccaaaaaaactcagctgcagctggaacatctgctgctggatctgcagatgattctgaatggcattaacaactataaaaacccagagctgactgacatgctgacctttaaattttatatgccaaaaaaagccactgaactgaaacatctgcagtgcctggaagaagagctgaaaccactggaagaagtgctgaacgctgcacagagcaaaaactttcatctgagaccaagagatctgattagcaacattaatgtgattgtgctggaactgaaaggcagtgaaaccacctttatgtgtgaatatgcagatgaaactgccaccattgtggaatttctgaacagatggattacctttgctcagagcattattagcaccctgacc

SEQ ID NO: 17 - DNA, 399 bp, Artificial Sequence
gccccaactagcagcagcaccaaaaaaactcagctgcagctggaacatctgctgctggatctgcagatgattctgaatggcattaacaactataaaaacccagatctgactgagatgctgacctttaaattttatatgccaaaaaaagccactgaactgaaacatctgcagtgcctggaagaagaactgaaaccactggaagaagtgctgaaccaggcacagagcaaaaactttcatctgagaccaagagatctgattagcaacattaatgtgattgtgctggaactgaaaggcagtgaaaccacctttatgtgtgaatatgcagatgaaactgccaccattgtggaatttctgaacagatggattacctttgctcagagcattattagcaccctgacc

SEQ ID NO: 18 - DNA, 399 bp, Artificial Sequence
gccccaactagcagcagcaccaaaaaaactcagctgcagctggaacatctgctgctggatctgcagatgattctgaatggcattaacaactataaaaacccagggctgactgacatgctgacctttaacttttatatgccaaaaaaagccactgaactgaaacatctgcagtgcctggaagaagagctgaaaccactggaagaagtgctgaacttcgcacagagcaaaaactttcatctgagaccaagagatctgattagcaacattaatgtgattgtgctggaactgaaaggcagtgaaaccacctttatgtgtgaatatgcagatgaaactgccaccattgtggaatttctgaacagatggattacctttgctcagagcattattagcaccctgacc

SEQ ID NO: 19 - DNA, 399 bp, Artificial Sequence
gccccaactagcagcagcaccaaaaaaactcagctgcagctggaacatctgctgctggatctgcagatgattctgaatggcattaacaactataaaaacccagatctgactgagatgctgacctttaaattttatatgccaaaaaaagccactgaactgaaacatctgcagtgcctggaagaagaactgaaaccactggaagaagtgctgaactcggcacagagcaaaaactttcatctgagaccaagagatctgattagcaacattaatgtgattgtgctggaactgaaaggcagtgaaaccacctttatgtgtgaatatgcagatgaaactgccaccattgtggaatttctgaacagatggattacctttgctcagagcattattagcaccctgacc

SEQ ID NO: 20 - DNA, 399 bp, Artificial Sequence
gccccaactagcagcagcaccaaaaaaactcagctgcagctggaacatctgctgctggatctgcagatgattctgaatggcattaacaactataaaaacccagagctgactgacatgctgacctttaaattttatatgccaaaaaaagccactgaactgaaacatctgcagtgcctggaagaagaactgaaaccactggaagaagtgctgaacggtgcacagagcaaaaactttcatctgagaccaagagatctgattagcaacattaatgtgattgtgctggaactgaaaggcagtgaaaccacctttatgtgtgaatatgcagatgaaactgccaccattgtggaatttctgaacagatggattacctttgctcagagcattattagcaccctgacc

SEQ ID NO: 21 - DNA, 399 bp, Artificial Sequence
gccccaactagcagcagcaccaaaaaaactcagctgcagctggaacatctgctgctggatctgcagatgattctgaatggcattaacaactataaaaacccagatctgactgatatgctgacctttaaattttatatgccaaaaaaagccactgaactgaaacatctgcagtgcctggaagaagaactgaaaccactggaagaagtgctgaacgcggcacagagcaaaaactttcatctgagaccaagagatctgattagcaacattaatgtgattgtgctggaactgaaaggcagtgaaaccacctttatgtgtgaatatgcagatgaaactgccaccattgtggaatttctgaacagatggattacctttgctcagagcattattagcaccctgacc

SEQ ID NO: 22 - protein, 133 aa, Artificial Sequence
APTSSSTKKTQLQLEHLLLDLQMILNGINNYKNPXLTXMLTXXFXMPKKATELKHLQCLEEELKPLEEVLNXAQSKNFHLRPRDLISNINVIVLELKGSETTFMCEYADETATIVEFLNRWITFXQSIISTLT

SEQ ID NO: 23 - protein, 133 aa, Artificial Sequence
APTSSSTKKTQLQLEHLLLDLQMILNGINNYKNPLLTDMLTLHFYMPKKATELKHLQCLEEELKPLEEVLNFAQSKNFHLRPRDLISNINVIVLELKGSETTFMCEYADETATIVEFLNRWITFCQSIISTLT

SEQ ID NO: 24 - protein, 133 aa, Artificial Sequence
APTSSSTKKTQLQLEHLLLDLQMILNGINNYKNPMLTDMLTVGFFMPKKATELKHLQCLEEELKPLEEVLNFAQSKNFHLRPRDLISNINVIVLELKGSETTFMCEYADETATIVEFLNRWITFCQSIISTLT

SEQ ID NO: 25 - protein, 133 aa, Artificial Sequence
APTSSSTKKTQLQLEHLLLDLQMILNGINNYKNPELTDMLTFKFYMPKKATELKHLQCLEEELKPLEEVLNAAQSKNFHLRPRDLISNINVIVLELKGSETTFMCEYADETATIVEFLNRWITFCQSIISTLT

SEQ ID NO: 26 - protein, 133 aa, Artificial Sequence
APTSSSTKKTQLQLEHLLLDLQMILNGINNYKNPGLTDMLTIQFFMPKKATELKHLQCLEEELKPLEEVLNFAQSKNFHLRPRDLISNINVIVLELKGSETTFMCEYADETATIVEFLNRWITFCQSIISTLT

SEQ ID NO: 27 - protein, 133 aa, Artificial Sequence
APTSSSTKKTQLQLEHLLLDLQMILNGINNYKNPSLTDMLTLQFYMPKKATELKHLQCLEEELKPLEEVLNFAQSKNFHLRPRDLISNINVIVLELKGSETTFMCEYADETATIVEFLNRWITFCQSIISTLT

SEQ ID NO: 28 - protein, 133 aa, Artificial Sequence
APTSSSTKKTQLQLEHLLLDLQMILNGINNYKNPDLTDMLTLRFFMPKKATELKHLQCLEEELKPLEEVLNFAQSKNFHLRPRDLISNINVIVLELKGSETTFMCEYADETATIVEFLNRWITFCQSIISTLT

SEQ ID NO: 29 - protein, 133 aa, Artificial Sequence
APTSSSTKKTQLQLEHLLLDLQMILNGINNYKNPDLTEMLTFKFYMPKKATELKHLQCLEEELKPLEEVLNQAQSKNFHLRPRDLISNINVIVLELKGSETTFMCEYADETATIVEFLNRWITFCQSIISTLT

SEQ ID NO: 30 - protein, 133 aa, Artificial Sequence
APTSSSTKKTQLQLEHLLLDLQMILNGINNYKNPYLTDMLTLGFYMPKKATELKHLQCLEEELKPLEEVLNFAQSKNFHLRPRDLISNINVIVLELKGSETTFMCEYADETATIVEFLNRWITFCQSIISTLT

SEQ ID NO: 31 - protein, 133 aa, Artificial Sequence
APTSSSTKKTQLQLEHLLLDLQMILNGINNYKNPGLTDMLTFNFYMPKKATELKHLQCLEEELKPLEEVLNFAQSKNFHLRPRDLISNINVIVLELKGSETTFMCEYADETATIVEFLNRWITFCQSIISTLT

SEQ ID NO: 32 - protein, 133 aa, Artificial Sequence
APTSSSTKKTQLQLEHLLLDLQMILNGINNYKNPGLTDMLTYSFDMPKKATELKHLQCLEEELKPLEEVLNLAQSKNFHLRPRDLISNINVIVLELKGSETTFMCEYADETATIVEFLNRWITFCQSIISTLT

SEQ ID NO: 33 - protein, 133 aa, Artificial Sequence
APTSSSTKKTQLQLEHLLLDLQMILNGINNYKNPDLTEMLTFKFYMPKKATELKHLQCLEEELKPLEEVLNSAQSKNFHLRPRDLISNINVIVLELKGSETTFMCEYADETATIVEFLNRWITFCQSIISTLT

SEQ ID NO: 34 - protein, 133 aa, Artificial Sequence
APTSSSTKKTQLQLEHLLLDLQMILNGINNYKNPELTEMLTFKFYMPKKATELKHLQCLEEELKPLEEVLNAAQSKNFHLRPRDLISNINVIVLELKGSETTFMCEYADETATIVEFLNRWITFCQSIISTLT

SEQ ID NO: 35 - protein, 133 aa, Artificial Sequence
APTSSSTKKTQLQLEHLLLDLQMILNGINNYKNPELTDMLTFKFYMPKKATELKHLQCLEEELKPLEEVLNGAQSKNFHLRPRDLISNINVIVLELKGSETTFMCEYADETATIVEFLNRWITFCQSIISTLT

SEQ ID NO: 36 - protein, 133 aa, Artificial Sequence
APTSSSTKKTQLQLEHLLLDLQMILNGINNYKNPDLTDMLTFKFYMPKKATELKHLQCLEEELKPLEEVLNAAQSKNFHLRPRDLISNINVIVLELKGSETTFMCEYADETATIVEFLNRWITFCQSIISTLT

SEQ ID NO: 37 - protein, 133 aa, Artificial Sequence
APTSSSTKKTQLQLEHLLLDLQMILNGINNYKNPELTDMLTFKFYMPKKATELKHLQCLEEELKPLEEVLNAAQSKNFHLRPRDLISNINVIVLELKGSETTFMCEYADETATIVEFLNRWITFAQSIISTLT

SEQ ID NO: 38 - protein, 133 aa, Artificial Sequence
APTSSSTKKTQLQLEHLLLDLQMILNGINNYKNPDLTEMLTFKFYMPKKATELKHLQCLEEELKPLEEVLNQAQSKNFHLRPRDLISNINVIVLELKGSETTFMCEYADETATIVEFLNRWITFAQSIISTLT

SEQ ID NO: 39 - protein, 133 aa, Artificial Sequence
APTSSSTKKTQLQLEHLLLDLQMILNGINNYKNPGLTDMLTFNFYMPKKATELKHLQCLEEELKPLEEVLNFAQSKNFHLRPRDLISNINVIVLELKGSETTFMCEYADETATIVEFLNRWITFAQSIISTLT

SEQ ID NO: 40 - protein, 133 aa, Artificial Sequence
APTSSSTKKTQLQLEHLLLDLQMILNGINNYKNPDLTEMLTFKFYMPKKATELKHLQCLEEELKPLEEVLNSAQSKNFHLRPRDLISNINVIVLELKGSETTFMCEYADETATIVEFLNRWITFAQSIISTLT

SEQ ID NO: 41 - protein, 133 aa, Artificial Sequence
APTSSSTKKTQLQLEHLLLDLQMILNGINNYKNPELTDMLTFKFYMPKKATELKHLQCLEEELKPLEEVLNGAQSKNFHLRPRDLISNINVIVLELKGSETTFMCEYADETATIVEFLNRWITFAQSIISTLT

SEQ ID NO: 42 - protein, 133 aa, Artificial Sequence
APTSSSTKKTQLQLEHLLLDLQMILNGINNYKNPDLTDMLTFKFYMPKKATELKHLQCLEEELKPLEEVLNAAQSKNFHLRPRDLISNINVIVLELKGSETTFMCEYADETATIVEFLNRWITFAQSIISTLT